European Patent Application EP 4 378 529 A1, published June 5, 2024. Title: ANTIBODY FOR USE IN A THERAPY INVOLVING EFFECTOR CELL ENGAGEMENT. Applicant: UNIVERSITÄTSKLINIKUM HAMBURG-EPPENDORF (UKE). The sequence listing filed with the application follows.

SEQUENCE LISTING (4 sequences)

SEQ ID NO: 1 - DNA, 1620 bp, synthetic construct
  source 1..1620: mol_type = other DNA
atgggatggagctgtatcatcctcttcttggtagcaacagctacaggcgcgcactccatggaagtgaagctgctggaatctggcggcggactggttcaacctggcggatctctgaagctgagctgtgccgccagcggcttcgacttcagcagatactggatgagctgggtccgacaggcccctggcaaaggactggaatggatcggcgagatcaaccccaccagcagcaccatcaacttcacccctagcctgaaggacaaggtgttcatcagccgggacaacgccaagaacaccctgtacctgcagatgagcaaagtgcggagcgaggacacagccctgtactactgtgccagaggcaactactacagatacggcgacgctatggactactggggccagggaacaagcgtgaccgtgtctaagatttctggcggaggcggatcaggcggcggaggaagcggtggcggaggatcaggtggtggtggatcaggcggaggtggcagctctgatatcgtgctgacacagtctccagccagcctggccgtttctctgggacagagagccaccatcagctgcagagccagcaagagcgtgtccacaagcggctacagctacctgcactggtatcagcagaagcccggccagcctcctaagctgctgatctacctggccagcaacctggaaagcggagtgcctgccagattttctggcagcggctctggcaccgacttcaccctgaatatccatcctgtggaagaagaggacgccgccacctactactgccagcacagtagagagctgcccttcacattcggcagcggcaccaagctggaaatcaaagcggccgcttcttctggtggcggcggaagcgatatcaagctccagcaatctggcgccgagctggctagacctggcgcctctgtgaagatgagctgcaagaccagcggctacaccttcaccagatacaccatgcactgggtcaagcagaggccaggccaaggcttggagtggatcggctacatcaaccccagccggggctacaccaactacaaccagaagttcaaggacaaggccacactgaccaccgacaagagcagcagcacagcctacatgcagctgagcagcctgaccagcgaagatagcgccgtgtactactgcgcccggtactacgacgatcactactgcctggattactggggccagggcacaaccctgacagtgtcatctgtggaaggcggctctggtggcagtggtggaagcggaggatctggcggagtggacgatatccagctgacacagagccccgccatcatgagtgctagccctggcgagaaagtgaccatgacctgtagagccagcagcagcgtgtcctacatgaactggtatcagcagaagtccggcacaagccccaagcggtggatctacgatacaagcaaggtggccagcggcgtgccctacagattttctggctctggcagcggcaccagctactccctgacaatcagcagcatggaagccgaggacgccgccacttactactgccagcagtggtctagcaaccctctgacctttggagccggcaccaagctggaactgaagcaccaccaccatcaccactaa

SEQ ID NO: 2 - protein, 539 aa, synthetic construct
MGWSCIILFLVATATGAHSMEVKLLESGGGLVQPGGSLKLSCAASGFDFSRYWMSWVRQAPGKGLEWIGEINPTSSTINFTPSLKDKVFISRDNAKNTLYLQMSKVRSEDTALYYCARGNYYRYGDAMDYWGQGTSVTVSKISGGGGSGGGGSGGGGSGGGGSGGGGSSDIVLTQSPASLAVSLGQRATISCRASKSVSTSGYSYLHWYQQKPGQPPKLLIYLASNLESGVPARFSGSGSGTDFTLNIHPVEEEDAATYYCQHSRELPFTFGSGTKLEIKAAASSGGGGSDIKLQQSGAELARPGASVKMSCKTSGYTFTRYTMHWVKQRPGQGLEWIGYINPSRGYTNYNQKFKDKATLTTDKSSSTAYMQLSSLTSEDSAVYYCARYYDDHYCLDYWGQGTTLTVSSVEGGSGGSGGSGGSGGVDDIQLTQSPAIMSASPGEKVTMTCRASSSVSYMNWYQQKSGTSPKRWIYDTSKVASGVPYRFSGSGSGTSYSLTISSMEAEDAATYYCQQWSSNPLTFGAGTKLELKHHHHHH

SEQ ID NO: 3 - DNA, 1617 bp, synthetic construct
  source 1..1617: mol_type = other DNA
atgggatggagctgtatcatcctcttcttggtagcaacagctacaggcgcgcactccatggaagtgaagctgctggaatctggcggcggactggttcaacctggcggatctctgaagctgagctgtgccgccagcggcttcgacttcagcagatactggatgagctgggtccgacaggcccctggcaaaggactggaatggatcggcgagatcaaccccaccagcagcaccatcaacttcacccctagcctgaaggacaaggtgttcatcagccgggacaacgccaagaacaccctgtacctgcagatgagcaaagtgcggagcgaggacacagccctgtactactgtgccagaggcaactactacagatacggcgacgctatggactactggggccagggaacaagcgtgaccgtgtctaagatttctggcggaggcggatcaggcggcggaggaagcggtggcggaggatcaggtggtggtggatcaggcggaggtggcagctctgatatcgtgctgacacagtctccagccagcctggccgtttctctgggacagagagccaccatcagctgcagagccagcaagagcgtgtccacaagcggctacagctacctgcactggtatcagcagaagcccggccagcctcctaagctgctgatctacctggccagcaacctggaaagcggagtgcctgccagattttctggcagcggctctggcaccgacttcaccctgaatatccatcctgtggaagaagaggacgccgccacctactactgccagcacagtagagagctgcccttcacattcggcagcggcaccaagctggaaatcaaagcggccgctggaggagggggatcaggaggcgggagcgaagtgcagttggtcgagtcagggggcgagctggtgcaacccggtggttcactccggctttcctgtgccgcctctggtctgacttttagctcttataacatggggtggttcaggcgagcgcccggtaaggagcgggagttcgtcgcatctatcacctggtcaggtcgggacaccttttacgcggacagtgtgaaaggacgatttacaatctcaagggataatgcaaagaatacggtttacttgcaaatgtctagcttgaagcctgaggacactgccgtctactattgcgccgctaatccctggccagtggctgcgccgcggagtggcacttattgggggcaaggtacccaggtcaccgtgagttctggcggagggggatccggcggtggaagcgaggtccaacttgtagaatctgggggcggtctcgtccaacccggaaattcattgcgcctttcatgcgcagccagtgggtttactttcagttccttcgggatgtcatgggtaagacaagcaccaggtaaaggcttggagtgggtgtccagtatctctggctctggaagcgatacactttacgcggattccgtgaaaggacggtttacaatttcacgggataacgctaaaacaacattgtatctgcaaatgaactcacttcgacccgaggatacggcagtgtattattgtacaatagggggatcattgagtcgatcctcacaaggcaccctcgttacagtaagctcctaa

SEQ ID NO: 4 - protein, 538 aa, synthetic construct
MGWSCIILFLVATATGAHSMEVKLLESGGGLVQPGGSLKLSCAASGFDFSRYWMSWVRQAPGKGLEWIGEINPTSSTINFTPSLKDKVFISRDNAKNTLYLQMSKVRSEDTALYYCARGNYYRYGDAMDYWGQGTSVTVSKISGGGGSGGGGSGGGGSGGGGSGGGGSSDIVLTQSPASLAVSLGQRATISCRASKSVSTSGYSYLHWYQQKPGQPPKLLIYLASNLESGVPARFSGSGSGTDFTLNIHPVEEEDAATYYCQHSRELPFTFGSGTKLEIKAAAGGGGSGGGSEVQLVESGGELVQPGGSLRLSCAASGLTFSSYNMGWFRRAPGKEREFVASITWSGRDTFYADSVKGRFTISRDNAKNTVYLQMSSLKPEDTAVYYCAANPWPVAAPRSGTYWGQGTQVTVSSGGGGSGGGSEVQLVESGGGLVQPGNSLRLSCAASGFTFSSFGMSWVRQAPGKGLEWVSSISGSGSDTLYADSVKGRFTISRDNAKTTLYLQMNSLRPEDTAVYYCTIGGSLSRSSQGTLVTVSS